European Patent Application EP 4 219 806 A2, published August 2, 2023. Title: Adeno-Associated Virus Library. Applicant: Ruprecht-Karls-Universität Heidelberg. Application EP. The sequence listing filed with the application follows.

SEQUENCE LISTING (52 sequences)

SEQ ID NO: 1-2 - skipped (2 entries)

SEQ ID NO: 3 - protein, 9 aa, synthetic construct
  REGION 1..9: note = inserted binding peptide
CDCRGDCFC

SEQ ID NO: 4 - protein, 7 aa, synthetic construct
  REGION 1..7: note = inserted binding peptide
NDVRSAN

SEQ ID NO: 5 - protein, 7 aa, synthetic construct
  REGION 1..7: note = inserted binding peptide
NDVRAVS

SEQ ID NO: 6 - protein, 7 aa, synthetic construct
  REGION 1..7: note = inserted binding peptide
MPLGAAG

SEQ ID NO: 7 - protein, 7 aa, synthetic construct
  REGION 1..7: note = inserted binding peptide
NYSRGVD

SEQ ID NO: 8 - protein, 7 aa, synthetic construct
  REGION 1..7: note = inserted binding peptide
NEARVRE

SEQ ID NO: 9 - protein, 11 aa, synthetic construct
  REGION 1..11: note = binding peptide
GCDCRGDCFCA

SEQ ID NO: 10 - protein, 9 aa, synthetic construct
  REGION 1..9: note = binding peptide
GNDVRSANA

SEQ ID NO: 11 - protein, 9 aa, synthetic construct
  REGION 1..9: note = binding peptide
GNDVRAVSA

SEQ ID NO: 12 - protein, 9 aa, synthetic construct
  REGION 1..9: note = binding peptide
GMPLGAAGA

SEQ ID NO: 13 - protein, 9 aa, synthetic construct
  REGION 1..9: note = binding peptide
GNYSRGVDA

SEQ ID NO: 14 - protein, 9 aa, synthetic construct
  REGION 1..9: note = binding peptide
GNEARVREA

SEQ ID NO: 15 - protein, 6 aa, synthetic construct
  REGION 1..6: note = Variant 1 insertion site AAV1 and AAV6
  REGION 3..4: note = MISC_FEATURE - insertion site
STDPAT

SEQ ID NO: 16 - protein, 6 aa, synthetic construct
  REGION 1..6: note = Variant 1 insertion site AAV2
  REGION 3..4: note = MISC_FEATURE - insertion site
GNRQAA

SEQ ID NO: 17 - protein, 6 aa, synthetic construct
  REGION 1..6: note = Variant 1 insertion site AAV3b
  REGION 3..4: note = MISC_FEATURE - insertion site
LQSSNT

SEQ ID NO: 18 - protein, 6 aa, synthetic construct
  REGION 1..6: note = Variant 1 insertion site AAV4
  REGION 3..4: note = MISC_FEATURE - insertion site
DQSNSN

SEQ ID NO: 19 - protein, 6 aa, synthetic construct
  REGION 1..6: note = Variant 1 insertion site AAV5
  REGION 3..4: note = MISC_FEATURE - insertion site
NQSSTT

SEQ ID NO: 20 - protein, 6 aa, synthetic construct
  REGION 1..6: note = Variant 1 insertion site AAV7
  REGION 3..4: note = MISC_FEATURE - insertion site
AANTAA

SEQ ID NO: 21 - protein, 6 aa, synthetic construct
  REGION 1..6: note = Variant 1 insertion site AAV8
  REGION 3..4: note = MISC_FEATURE - insertion site
QQNTAP

SEQ ID NO: 22 - protein, 6 aa, synthetic construct
  REGION 1..6: note = Variant 1 insertion site AAV9
  REGION 3..4: note = MISC_FEATURE - insertion site
SAQAQA

SEQ ID NO: 23 - protein, 6 aa, synthetic construct
  REGION 1..6: note = Variant 1 insertion site AAVrh10
  REGION 3..4: note = MISC_FEATURE - insertion site
QQNAAP

SEQ ID NO: 24 - protein, 6 aa, synthetic construct
  REGION 1..6: note = Variant 1 insertion site AAVpo.1
  REGION 3..4: note = MISC_FEATURE - insertion site
NQNSNT

SEQ ID NO: 25 - protein, 6 aa, synthetic construct
  REGION 1..6: note = Variant 1 insertion site AAV12
  REGION 3..4: note = MISC_FEATURE - insertion site
NQNATT

SEQ ID NO: 26 - protein, 6 aa, synthetic construct
  REGION 1..6: note = Variant 2 insertion site AAV1 and AAV6
  REGION 3..4: note = MISC_FEATURE - insertion site
SSSTDP

SEQ ID NO: 27 - protein, 6 aa, synthetic construct
  REGION 1..6: note = Variant 2 insertion site AAV2
  REGION 3..4: note = MISC_FEATURE - insertion site
RGNRQA

SEQ ID NO: 28 - protein, 6 aa, synthetic construct
  REGION 1..6: note = Variant 2 insertion site AAV3b
  REGION 3..4: note = MISC_FEATURE - insertion site
SSNTAP

SEQ ID NO: 29 - protein, 6 aa, synthetic construct
  REGION 1..6: note = Variant 2 insertion site AAV4
  REGION 3..4: note = MISC_FEATURE - insertion site
SNSNLP

SEQ ID NO: 30 - protein, 6 aa, synthetic construct
  REGION 1..6: note = Variant 2 insertion site AAV5
  REGION 3..4: note = MISC_FEATURE - insertion site
SSTTAP

SEQ ID NO: 31 - protein, 6 aa, synthetic construct
  REGION 1..6: note = Variant 2 insertion site AAVpo.1
  REGION 3..4: note = MISC_FEATURE - insertion site
NSNTHP

SEQ ID NO: 32 - protein, 6 aa, synthetic construct
  REGION 1..6: note = Variant 2 insertion site AAV12
  REGION 3..4: note = MISC_FEATURE - insertion site
NATTAP

SEQ ID NO: 33 - protein, 11 aa, synthetic construct
  REGION 1..11: note = AAV2 wt insertion site
  REGION 5..6: note = MISC_FEATURE - insertion site
TNLQRGNRQAA

SEQ ID NO: 34 - DNA, 33 bp, synthetic construct
  misc_feature 1..33: note = AAV2 wt insertion site encoding
  source 1..33: mol_type = other DNA
accaacctccagagaggcaacagacaagcagct

SEQ ID NO: 35 - protein, 12 aa, synthetic construct
  REGION 1..12: note = AAV2 NIS
  REGION 7..8: note = MISC_FEATURE - insertion site
TNLQGQRGAQAA

SEQ ID NO: 36 - DNA, 36 bp, synthetic construct
  misc_feature 1..36: note = AAV2 NIS encoding
  source 1..36: mol_type = other DNA
accaacctccagggccagagaggcgcccaggcggcc

SEQ ID NO: 37 - protein, 13 aa, synthetic construct
  REGION 1..13: note = AAV2 2xA
  REGION 10..11: note = MISC_FEATURE - insertion site
TNLQRGNAAAAAR

SEQ ID NO: 38 - DNA, 39 bp, synthetic construct
  misc_feature 1..39: note = AAV2 2xA encoding
  source 1..39: mol_type = other DNA
accaacctccagagaggcaacgcggcggcagcagccaga

SEQ ID NO: 39 - protein, 14 aa, synthetic construct
  REGION 1..14: note = AAV2 3xA
  REGION 10..11: note = MISC_FEATURE - insertion site
TNLQRGNAAAAAAR

SEQ ID NO: 40 - DNA, 42 bp, synthetic construct
  misc_feature 1..42: note = AAV2 3xA encoding
  source 1..42: mol_type = other DNA
accaacctccagagaggcaacgcggcggcagcagccgcgaga

SEQ ID NO: 41 - protein, 15 aa, synthetic construct
  REGION 1..15: note = AAV2 4xA
  REGION 10..11: note = MISC_FEATURE - insertion site
TNLQRGNAAAAAAAR

SEQ ID NO: 42 - DNA, 45 bp, synthetic construct
  misc_feature 1..45: note = AAV2 4xA encoding
  source 1..45: mol_type = other DNA
accaacctccagagaggcaacgcggcggcagcagccgcggccaga

SEQ ID NO: 43 - protein, 16 aa, synthetic construct
  REGION 1..16: note = AAV2 wt extended
TNLQRGNRQAATADVN

SEQ ID NO: 44 - protein, 25 aa, synthetic construct
  REGION 1..25: note = AAV2_A2(OIS)
TNLQRGQRGNYSRGVDAQAATADVN

SEQ ID NO: 45 - protein, 25 aa, synthetic construct
  REGION 1..25: note = AAV2_A2(NIS)
TNLQGQRGNYSRGVDAQAAATADVN

SEQ ID NO: 46 - protein, 28 aa, synthetic construct
  REGION 1..28: note = AAV2_A2_2xA(NIS)
TNLQRGNAAANYSRGVDAARQAATADVN

SEQ ID NO: 47 - protein, 29 aa, synthetic construct
  REGION 1..29: note = AAV2_A2_3xA(NIS)
TNLQRGNAAANYSRGVDAAARQAATADVN

SEQ ID NO: 48 - protein, 30 aa, synthetic construct
  REGION 1..30: note = AAV2_A2_4xA(NIS)
TNLQRGNAAANYSRGVDAAAARQAATADVN

SEQ ID NO: 49 - protein, 7 aa, synthetic construct
  REGION 1..7: note = inserted binding peptide
NSSRDLG

SEQ ID NO: 50 - protein, 7 aa, synthetic construct
  REGION 1..7: note = inserted binding peptide
SEGLKNL

SEQ ID NO: 51 - protein, 7 aa, synthetic construct
  REGION 1..7: note = inserted binding peptide
PSVPRPP

SEQ ID NO: 52 - protein, 7 aa, synthetic construct
  REGION 1..7: note = inserted binding peptide
NFTRLSA